European Patent Application EP 4 501 953 A1, published February 5, 2025. Title: 特异性结合CD7的抗体及其在制备嵌合抗原受体中的应用. Applicant: 中国医学科学院血液病医院（中国医学科学院血液学研究所）. Application WO. The sequence listing filed with the application follows.

SEQUENCE LISTING (12 sequences)

SEQ ID NO: 1 - protein, 15 aa, synthetic construct
RASKSVSASGYSYMH

SEQ ID NO: 2 - protein, 7 aa, synthetic construct
LASNLES

SEQ ID NO: 3 - protein, 9 aa, synthetic construct
QHSRELPYT

SEQ ID NO: 4 - protein, 12 aa, synthetic construct
GISITTGNYRWS

SEQ ID NO: 5 - protein, 16 aa, synthetic construct
YIYYSGIITYNPSRTS

SEQ ID NO: 6 - protein, 14 aa, synthetic construct
ERGIYYDSLWYFDV

SEQ ID NO: 7 - protein, 113 aa, synthetic construct
DIVLTQSPASLAVSLGQRATISCRASKSVSASGYSYMHWYQQKPGQPPKLLIYLASNLESGVPARFSGSGSGTDFTLNIHPVEEEDAVTYYCQHSRELPYTFGGGTKLEIKRA

SEQ ID NO: 8 - protein, 124 aa, synthetic construct
QVQLQESGPGLVKPSQTVSLTCTVTGISITTGNYRWSWIRQFPGNKLEWIGYIYYSGIITYNPSRTSRTTITRDISKNQFFLEMNSLTAEDTATYYCARERGIYYDSLWYFDVWGAGTTVTVSS

SEQ ID NO: 9 - protein, 252 aa, synthetic construct
DIVLTQSPASLAVSLGQRATISCRASKSVSASGYSYMHWYQQKPGQPPKLLIYLASNLESGVPARFSGSGSGTDFTLNIHPVEEEDAVTYYCQHSRELPYTFGGGTKLEIKRAGGGGSGGGGSGGGGSQVQLQESGPGLVKPSQTVSLTCTVTGISITTGNYRWSWIRQFPGNKLEWIGYIYYSGIITYNPSRTSRTTITRDISKNQFFLEMNSLTAEDTATYYCARERGIYYDSLWYFDVWGAGTTVTVSS

SEQ ID NO: 10 - protein, 21 aa, synthetic construct
MALPVTALLLPLALLLHAARP

SEQ ID NO: 11 - protein, 500 aa, synthetic construct
MALPVTALLLPLALLLHAARPASDIVLTQSPASLAVSLGQRATISCRASKSVSASGYSYMHWYQQKPGQPPKLLIYLASNLESGVPARFSGSGSGTDFTLNIHPVEEEDAVTYYCQHSRELPYTFGGGTKLEIKRAGGGGSGGGGSGGGGSQVQLQESGPGLVKPSQTVSLTCTVTGISITTGNYRWSWIRQFPGNKLEWIGYIYYSGIITYNPSRTSRTTITRDISKNQFFLEMNSLTAEDTATYYCARERGIYYDSLWYFDVWGAGTTVTVSSEFTTTPAPRPPTPAPTIASQPLSLRPEACRPAAGGAVHTRGLDFACDIYIWAPLAGTCGVLLLSLVITLYCKRGRKKLLYIFKQPFMRPVQTTQEEDGCSCRFPEEEEGGCELRVKFSRSADAPAYQQGQNQLYNELNLGRREEYDVLDKRRGRDPEMGGKPRRKNPQEGLYNELQKDKMAEAYSEIGMKGERRRGKGHDGLYQGLSTATKDTYDALHMQALPPR

SEQ ID NO: 12 - DNA, 1500 bp, synthetic construct
  source 1..1500: mol_type = other DNA
atggccttaccagtgaccgccttgctcctgccgctggccttgctgctccacgccgccaggccggctagcgacattgtgctgacacagtctcctgcttccttagctgtatctctggggcagagggccaccatctcatgcagggccagcaaaagtgtcagtgcatctggctatagttatatgcactggtaccaacagaaaccaggacagccacccaaactcctcatctatcttgcatccaacctagaatctggggtccctgccaggttcagtggcagtgggtctgggacagacttcaccctcaacatccatcctgtggaggaggaggatgctgtaacctattactgtcagcacagtagggagcttccgtacacgttcggaggggggaccaagctggaaataaaacgggctggtggtggtggttctggcggcggcggctccggtggtggtggttctcaggtgcagctgcaggagtcaggacctggtctggtgaaaccttctcagacagtgtccctcacctgcactgtcactggcatctccatcaccactggaaattacagatggagctggatccggcagtttccaggaaacaaactggagtggatagggtacatatactacagtggaatcattacctataatccatctcgcacaagtcgaaccaccatcactagagacatttccaagaaccaattcttcctggaaatgaactctttgactgctgaagacacagccacatactactgtgcacgagagagagggatctactatgattccctatggtacttcgatgtctggggcgcagggaccacggtcaccgtctcttcagaattcaccacgacgccagcgccgcgaccaccaacaccggcgcccaccatcgcgtcgcagcccctgtccctgcgcccagaggcgtgccggccagcggcggggggcgcagtgcacacgagggggctggacttcgcctgtgatatctacatctgggcgcccttggccgggacttgtggggtccttctcctgtcactggttatcaccctttactgcaaacggggcagaaagaaactcctgtatatattcaaacaaccatttatgagaccagtacaaactactcaagaggaagatggctgtagctgccgatttccagaagaagaagaaggaggatgtgaactgagagtgaagttcagcaggagcgcagacgcccccgcgtaccagcagggccagaaccagctctataacgagctcaatctaggacgaagagaggagtacgatgttttggacaagagacgtggccgggaccctgagatggggggaaagccgagaaggaagaaccctcaggaaggcctgtacaatgaactgcagaaagataagatggcggaggcctacagtgagattgggatgaaaggcgagcgccggaggggcaaggggcacgatggcctttaccagggtctcagtacagccaccaaggacacctacgacgcccttcacatgcaggccctgccccctcgc